European Patent Specification EP 4 326 339 B1, published April 2, 2025. Title: Compositions and methods for treating retinal degenerative disorders. Applicant: SPARINGVISION INSERM SORBONNE UNIVERSITE CNRS. The sequence listing filed with the application follows.

SEQUENCE LISTING (37 sequences)

SEQ ID NO: 1 - protein, 109 aa, Homo sapiens
MASLFSGRILIRNNSDQDELDTEAEVSRRLENRLVLLFFGAGACPQCQAFVPILKDFFVRLTDEFYVLRAAQLALVYVSQDSTEEQQDLFLKDMPKKWLFLPFEDDLRR

SEQ ID NO: 2 - protein, 212 aa, Homo sapiens
MASLFSGRILIRNNSDQDELDTEAEVSRRLENRLVLLFFGAGACPQCQAFVPILKDFFVRLTDEFYVLRAAQLALVYVSQDSTEEQQDLFLKDMPKKWLFLPFEDDLRRDLGRQFSVERLPAVVVLKPDGDVLTRDGADEIQRLGTACFANWQEAAEVLDRNFQLPEDLEDQEPRSLTECLRRHKYRVEKAARGGRDPGGGGGEEGGAGGLF

SEQ ID NO: 3 - DNA, 330 bp, Homo sapiens
atggcctccctgttctctggccgcatcctgatccgcaacaatagcgaccaggacgagctggatacggaggctgaggtcagtcgcaggctggagaaccggctggtgctgctgttctttggtgctggggcttgtccacagtgccaggccttcgtgcccatcctcaaggacttcttcgtgcggctcacagatgagttctatgtactgcgggcggctcagctggccctggtgtacgtgtcccaggactccacggaggagcagcaggacctgttcctcaaggacatgccaaagaaatggcttttcctgccctttgaggatgatctgaggaggtga

SEQ ID NO: 4 - DNA, 330 bp, Pan troglodytes
atggcctccctgttctctggccgcatcctgatccgcaacaatagcgaccaggacgaactggatacggaggctgaggtcagtcgcaggctggagaaccggctggtgctgctgttctttggtgccggggcttgtccacagtgccaggccttcgtgcccatcctcaaggacttcttcgtgcggctcacagatgagttctatgtactgcgggcggctcagctggccctggtgtacgtgtcccaggactccacggaggagcagcaggacctgttcctcaaggacatgccaaagaagtggcttttcctgccctttgaggatgatctgaggaggtga

SEQ ID NO: 5 - DNA, 639 bp, Homo sapiens
atggcctccctgttctctggccgcatcctgatccgcaacaatagcgaccaggacgagctggatacggaggctgaggtcagtcgcaggctggagaaccggctggtgctgctgttctttggtgctggggcttgtccacagtgccaggccttcgtgcccatcctcaaggacttcttcgtgcggctcacagatgagttctatgtactgcgggcggctcagctggccctggtgtacgtgtcccaggactccacggaggagcagcaggacctgttcctcaaggacatgccaaagaaatggcttttcctgccctttgaggatgatctgaggagggacctcgggcgccagttctcagtggagcgcctgccggcggtcgtggtgctcaagccggacggggacgtgctcactcgcgacggcgccgacgagatccagcgcctgggcaccgcctgcttcgccaactggcaggaggcggccgaggtgctggaccgcaacttccagctgccagaggacctggaggaccaggagccacggagcctcaccgagtgcctgcgccgccacaagtaccgcgtggaaaaggcggcgcgaggcgggcgcgaccccgggggagggggtggggaggagggcggggccggggggctgttctga

SEQ ID NO: 6 - DNA, 330 bp, Homo sapiens
atggcctccttgttctccggccgaatcctgatccgaaacaatagtgaccaggatgagctggatacagaagctgaggtcagtcgcagactggagaacaggctggtccttctgttctttggtgctggggcttgtcctcagtgccaggccttcgtgcccatcctcaaggacttctttgtgcggctcacggatgagttctatgtactgcgggcagctcaactggctctagtatatgtgtcacaggactccactgaggagcagcaggacctcttcctgaaggacatgccaaagaaatggcttttcctgccctttgaggatgatctgaggaggtag

SEQ ID NO: 7 - DNA, 330 bp, Artificial sequence
  optimized cDNA hRdCVF
atggccagcctcttctccggacgcatcctgattcgcaacaattccgaccaagacgaactggataccgaggccgaagtctcgcggagattggagaacaggcttgtgctgctgttctttggcgcgggagcgtgtcctcagtgccaggctttcgtgccaatcctgaaggatttcttcgtgcggctgactgacgaattctacgtcctccgggccgcccagctggcactggtgtacgtgtcccaagactcaaccgaggaacagcaggatctgttcctcaaggacatgcccaaaaagtggctgttcctgccgtttgaggacgacttgcggcgctag

SEQ ID NO: 8 - DNA, 639 bp, Artificial sequence
  optimized cDNA hRdCVFL
atggcctcactgttctccgggcgcatcctcatccgaaacaacagcgatcaggacgaattggacaccgaggctgaagtctcccgccggctggaaaacaggctcgtgctcctgttcttcggtgccggagcgtgcccgcagtgccaagccttcgtcccaattcttaaggacttctttgtgcgcctcactgatgagttttacgtgctccgggcagcgcagctggccttggtgtatgtgtcgcaagattccactgaggaacaacaggacctgttcctgaaagacatgcctaagaagtggcttttcctgcccttcgaggacgacctgagaagggacctgggacgccagttcagcgtggaacggctgccggccgtcgtggtgctgaagcccgacggggacgtgcttacccgggatggcgctgacgaaatccagaggctgggcaccgcctgtttcgcaaattggcaggaggccgccgaagtgctcgaccggaacttccagctgcccgaggatctggaggaccaggaacctcggtccctgaccgagtgcctcagacgccacaagtaccgcgtggaaaaggccgcgagaggaggacgggacccgggtggcgggggaggcgaagagggcggagccggtggcctgttctga

SEQ ID NO: 9 - protein, 423 aa, Homo sapiens
MAKLTESMTNVLEGDSMDQDVESPVAIHQPKLPKQARDDLPRHISRDRTKRKIQRYVRKDGKCNVHHGNVRETYRYLTDIFTTLVDLKWRFNLLIFVMVYTVTWLFFGMIWWLIAYIRGDMDHIEDPSWTPCVTNLNGFVSAFLFSIETETTIGYGYRVITDKCPEGIILLLIQSVLGSIVNAFMVGCMFVKISQPKKRAETLVFSTHAVISMRDGKLCLMFRVGDLRNSHIVEASIRAKLIKSKQTSEGEFIPLNQTDINVGYYTGDDRLFLVSPLIISHEINQQSPFWEISKAQLPKEELEIVVILEGMVEATGMTCQARSSYITSEILWGYRFTPVLTLEDGFYEVDYNSFHETYETSTPSLSAKELAELASRAELPLSWSVSSKLNQHAELETEEEEKNLEEQTERNGDVANLENESKV

SEQ ID NO: 10 - protein, 408 aa, Rattus norvegicus
MDQDVESPVAIHQPKLPKQARDDLPRHISRDRTKRRIQRYVRKDGKCNVHHGNVRETYRYLTDIFTTLVDLKWRFNLLIFVMVYTVTWLFFGMIWWLIAYIRGDMDHIEDPSWTPCVTNLNGFVSAFLFSIETETTIGYGYRVITDKCPEGIILLLIQSVLGSIVNAFMVGCMFVKISQPKKRAETLVFSTHAVISMRDGKLCLMFRVGDLRNSHIVEASIRAKLIKSKQTSEGEFIPLNQTDINVGYYTGDDRLFLVSPLIISHEINQQSPFWEISKAQLPKEELEIVVILEGMVEATGMTCQARSSYVTSEILWGYRFTPVLTLEDGFYEVDYNSFHETHETSTPSLSAKELAELANRAELPLSWSVSSKLNQHAELETEEEEKNPEELTERNGDVANLENESKVA

SEQ ID NO: 11 - protein, 425 aa, Mus musculus
MTMAKLTESMTNVLEGDSMDQDVESPVAIHQPKLPKQARDDLPRHISRDRTKRKIQRYVRKDGKCNVHHGNVRETYRYLTDIFTTLVDLKWRFNLLIFVMVYTVTWLFFGMIWWLIAYIRGDMDHIEDPSWTPCVTNLNGFVSAFLFSIETETTIGYGYRVITDKCPEGIILLLIQSVLGSIVNAFMVGCMFVKISQPKKRAETLVFSTHAVISMRDGKLCLMFRVGDLRNSHIVEASIRAKLIKSKQTSEGEFIPLNQTDINVGYYTGDDRLFLVSPLIISHEINQQSPFWEISKAQLPKEELEIVVILEGMVEATGMTCQARSSYITSEILWGYRFTPVLTLEDGFYEVDYNSFHETYETSTPSLSAKELAELANRAELPLSWSVSSKLNQHAELETEEEEKNPEELTERNGDVANLENESKV

SEQ ID NO: 12 - DNA, 1272 bp, Homo sapiens
atggccaagctgaccgagagcatgacaaatgtgctggagggcgacagcatggaccaggatgttgaaagccccgtggccatccaccagcctaagctgcctaaacaggccagggacgacctgcctagacacatcagcagagacaggaccaagcggaagatccagagatacgtgcggaaggacggcaagtgcaatgtgcaccacggcaacgtgcgggaaacctacagatacctgaccgacatcttcaccacactggtggacctgaagtggcggttcaacctgctgatcttcgtgatggtgtacacagtgacctggctgttcttcggcatgatctggtggctgatcgcctacatcagaggcgacatggaccacatcgaggaccctagctggaccccttgcgtgaccaacctgaatggcttcgtgtccgccttcctgttcagcatcgagacagagacaaccatcggctacggctacagagtgatcaccgacaagtgccctgagggcatcatcctgctgctgatccagtctgtgctgggcagcatcgtgaacgccttcatggtcggatgcatgttcgtgaagatctcccagccaaagaagcgggccgagacactggtgtttagcacccacgccgtgatcagcatgagagatggcaagctgtgcctgatgttcagagtgggcgacctgcggaacagccacatcgtggaagccagcatccgggccaaactgatcaagagcaagcagaccagcgagggcgagttcatccctctgaaccagaccgatatcaacgtgggctactacaccggcgacgacagactgtttctggtgtcccctctgatcatctcccacgagatcaaccagcagagccccttttgggagatcagcaaggcccagctgccaaaagaggaactggaaatcgtcgtgatcctggaaggcatggtggaagctaccggcatgacctgtcaggccagaagcagctacatcaccagcgagatcctgtggggctacagattcacccctgtgctgaccctggaagatggcttctacgaggtggactacaactccttccacgagacatacgagacaagcacccctagcctgagcgccaaagagctggctgaactggcctctagagccgagcttcctctgtcttggagcgtgtccagcaagctgaatcagcacgccgagctggaaaccgaggaagaggaaaagaacctggaagaacagaccgagcggaacggcgacgtggccaacctggaaaatgagagcaaggtgtag

SEQ ID NO: 13 - DNA, 798 bp, Gallus gallus domesticus
cgttacataacttacggtaaatggcccgcctggctgaccgcccaacgacccccgcccattgacgtcaatagtaacgccaatagggactttccattgacgtcaatgggtggagtatttacggtaaactgcccacttggcagtacatcaagtgtatcatatgccaagtacgccccctattgacgtcaatgacggtaaatggcccgcctggcattgtgcccagtacatgaccttatgggactttcctacttggcagtacatctacgtattagtcatcgctattaccatggtcgaggtgagccccacgttctgcttcactctccccatctcccccccctccccacccccaattttgtatttatttattttttaattattttgtgcagcgatgggggcggggggggggggggggcgcgcgccaggcggggcggggcggggcgaggggcggggcggggcgaggcggagaggtgcggcggcagccaatcagagcggcgcgctccgaaagtttccttttatggcgaggcggcggcggcggcggccctataaaaagcgaagcgcgcggcgggcgggagtcgctgcgcgctgccttcgccccgtgccccgctccgccgccgcctcgcgccgcccgccccggctctgactgaccgcgttactcccacaggtgagcgggcgggacggcccttctcctccgggctgtaattagctgagcaagaggtaagggtttaagggatggttggttggtggggtattaatgtttaattacctggagcacctgcctgaaatcactttttttcaggttgg

SEQ ID NO: 14 - DNA, 292 bp, Homo spaiens
gggccccagaagcctggtggttgtttgtccttctcaggggaaaagtgaggcggccccttggaggaaggggccgggcagaatgatctaatcggattccaagcagctcaggggattgtctttttctagcaccttcttgccactcctaagcgtcctccgtgaccccggctgggatttagcctggtgctgtgtcagccccggtctcccaggggcttcccagtggtccccaggaaccctcgacagggcccggtctctctcgtccagcaagggcagggacgggccacaggccaagggc

SEQ ID NO: 15 - DNA, 93 bp, artificial sequence
  GRK1-93 promoter
tctaatcggattccaagcagctcaggggattgtctttttctagcaccttcttgccactcctaagcgtcctccgtgaccccggctgggatttag

SEQ ID NO: 16 - DNA, 1727 bp, artificial sequence
  PR1.7 promoter
ggaggctgaggggtggggaaagggcatgggtgtttcatgaggacagagcttccgtttcatgcaatgaaaagagtttggagacggatggtggtgactggactatacacttacacacggtagcgatggtacactttgtattatgtatattttaccacgatctttttaaagtgtcaaaggcaaatggccaaatggttccttgtcctatagctgtagcagccatcggctgttagtgacaaagcccctgagtcaagatgacagcagcccccataactcctaatcggctctcccgcgtggagtcatttaggagtagtcgcattagagacaagtccaacatctaatcttccaccctggccagggccccagctggcagcgagggtgggagactccgggcagagcagagggcgctgacattggggcccggcctggcttgggtccctctggcctttccccaggggccctctttccttggggctttcttgggccgccactgctcccgctcctctccccccatcccaccccctcaccccctcgttcttcatatccttctctagtgctccctccactttcatccacccttctgcaagagtgtgggaccacaaatgagttttcacctggcctggggacacacgtgcccccacaggtgctgagtgactttctaggacagtaatctgctttaggctaaaatgggacttgatcttctgttagccctaatcatcaattagcagagccggtgaaggtgcagaacctaccgcctttccaggcctcctcccacctctgccacctccactctccttcctgggatgtgggggctggcacacgtgtggcccagggcattggtgggattgcactgagctgggtcattagcgtaatcctggacaagggcagacagggcgagcggagggccagctccggggctcaggcaaggctgggggcttcccccagacaccccactcctcctctgctggacccccacttcatagggcacttcgtgttctcaaagggcttccaaatagcatggtggccttggatgcccagggaagcctcagagttgcttatctccctctagacagaaggggaatctcggtcaagagggagaggtcgccctgttcaaggccacccagccagctcatggcggtaatgggacaaggctggccagccatcccaccctcagaagggacccggtggggcaggtgatctcagaggaggctcacttctgggtctcacattcttggatccggttccaggcctcggccctaaatagtctccctgggctttcaagagaaccacatgagaaaggaggattcgggctctgagcagtttcaccacccaccccccagtctgcaaatcctgacccgtgggtccacctgccccaaaggcggacgcaggacagtagaagggaacagagaacacataaacacagagagggccacagcggctcccacagtcaccgccaccttcctggcggggatgggtggggcgtctgagtttggttcccagcaaatccctctgagccgcccttgcgggctcgcctcaggagcaggggagcaagaggtgggaggaggaggtctaagtcccaggcccaattaagagatcaggtagtgtagggtttgggagcttttaaggtgaagaggcccgggctgatcccacaggccagtataaagcgccgtgaccctcaggtgatgcgccagggccggctgccgtcggggacagggctttccatagccatg

SEQ ID NO: 17 - DNA, 500 bp, artificial sequence
  ProA7 promoter
catcctgagagatgagccaggacaaagaaccagtaatagctcctggagcagcacatctgttttgccaggattatcccttggatctcttaaaaccgagaccttgtaatctgaagactcaacttgggctgtacccttaaccttcagctctatgatgcaagtgagtccacaggaccggaggctttgagatgagcttttcagaagggaggagttggccgcttgctcccagagctccagcacctgcattcttctggctatgtcagaagccagatcatttccctcgttaaaaacaaaaacaaaaaaacaaacaaacaaaatgttagtctttgccctttatctgcctggcaaagcttttaattggcttgatctgtcattccgctagacataaaggggacaatccccggattaggaaggagctctccagctcgggtaaggagtctcaaggcaaggtaggcaagcaccaccggtccgcactctcgcccagcttttacgggaagaagaga

SEQ ID NO: 18 - protein, 8 aa, artificial sequence
  core sequence motif of 2A-cleaving peptides
  misc_feature (2)..(2): Xaa can be any naturally occurring amino acid
  misc_feature (4)..(4): Xaa can be any naturally occurring amino acid
DXEXNPGP

SEQ ID NO: 19 - protein, 22 aa, artificial sequence
  P2A cleaving peptide
GSGATNFSLLKQAGDVEENPGP

SEQ ID NO: 20 - protein, 21 aa, artificial sequence
  T2A cleaving peptide
GSGEGRGSLLTCGDVEENPGP

SEQ ID NO: 21 - protein, 23 aa, artificial sequence
  E2A cleaving peptide
GSGQCTNYALLKLAGDVESNPGP

SEQ ID NO: 22 - protein, 25 aa, artificial sequence
  F2A cleaving peptide
GSGVKQTLNFDLLKLAGDVESNPGP

SEQ ID NO: 23 - DNA, 66 bp, artificial sequence
  cDNA encoding P2A cleaving peptide
ggaagcggagccacgaacttctctctgttaaagcaagcaggagatgttgaagaaaaccccgggcct

SEQ ID NO: 24 - DNA, 598 bp, Woodchuck Hepatitis Virus
cgataatcaacctctggattacaaaatttgtgaaagattgactggtattcttaactatgttgctccttttacgctatgtggatacgctgctttaatgcctttgtatcatgctattgcttcccgtatggctttcattttctcctccttgtataaatcctggttgctgtctctttatgaggagttgtggcccgttgtcaggcaacgtggcgtggtgtgcactgtgtttgctgacgcaacccccactggttggggcattgccaccacctgtcagctcctttccgggactttcgctttccccctccctattgccacggcggaactcatcgccgcctgccttgcccgctgctggacaggggctcggctgttgggcactgacaattccgtggtgttgtcggggaagctgacgtcctttccatggctgctcgcctgtgttgccacctggattctgcgcgggacgtccttctgctacgtcccttcggccctcaatccagcggaccttccttcccgcggcctgctgccggctctgcggcctcttccgcgtcttcgccttcgccctcagacgagtcggatctccctttgggccgcctccccgcatcgg

SEQ ID NO: 25 - protein, 7 aa, artificial sequence
  insertion peptide
LGETTRP

SEQ ID NO: 26 - protein, 7 aa, artificial sequence
  insertion peptide
NETITRP

SEQ ID NO: 27 - protein, 7 aa, artificial sequence
  insertion peptide
KAGQANN

SEQ ID NO: 28 - protein, 7 aa, artificial sequence
  insertion peptide
KDPKTTN

SEQ ID NO: 29 - protein, 7 aa, artificial sequence
  insertion peptide
KDTDTTR

SEQ ID NO: 30 - protein, 7 aa, artificial sequence
  insertion peptide
RAGGSVG

SEQ ID NO: 31 - protein, 7 aa, artificial sequence
  insertion peptide
AVDTTKF

SEQ ID NO: 32 - protein, 7 aa, artificial sequence
  insertion peptide
STGKVPN

SEQ ID NO: 33 - protein, 10 aa, artificial sequence
  insertion peptide
AALGETTRPA

SEQ ID NO: 34 - protein, 10 aa, artificial sequence
  insertion peptide
LALGETTRPA

SEQ ID NO: 35 - DNA, 1224 bp, Rattus norvegicus
atggaccaagacgtggaaagcccagtggccattcaccagccaaagttgcctaagcaggccagggatgacctgccaagacacatcagccgagacaggaccaaaaggagaatccagaggtacgtgaggaaggatgggaagtgtaacgtccaccacggcaacgtgcgggagacgtaccgatacctgacggacatcttcaccaccctggtggacctaaagtggagattcaacctattgatctttgtcatggtctacacagtgacgtggcttttctttgggatgatctggtggctaattgcatacatccggggagatatggaccacatagaggacccctcgtggactccctgtgttaccaacctcaacgggtttgtctccgcttttttattctcaatagagacagaaaccaccattggttatggctacagggtcatcacggacaagtgcccagaaggaattattctcctcttaatccagtccgtgttggggtccattgtcaacgccttcatggtaggatgtatgtttgtgaaaatatcccaacccaagaagagggcagagaccctggtcttttccacccatgcggtaatctccatgcgggatgggaaactatgcctgatgttccgggtaggggacttgaggaattcccacattgtggaggcctccatcagagccaagttgatcaagtccaaacagacttcagagggggagttcattcccctcaaccagacggatatcaacgtagggtactacaccggggatgaccgactctttctcgtgtcaccgctgattattagccatgaaattaaccaacagagtcccttctgggagatctccaaagcccagctgcctaaagaggaactggagattgtggtcatcctggagggaatggtggaagccacaggaatgacgtgccaagctcgaagctcctacgtcaccagtgagatcctgtggggttaccggttcacaccagtcctgacactggaggacgggttctatgaagttgactacaacagcttccatgagacccatgagaccagcaccccgtcccttagcgccaaagagctagccgagctggctaaccgggcagagctgcccctgagctggtctgtgtccagcaaactgaaccaacatgcagaactggagacggaagaggaagagaagaacccggaagaactgacagagaggaatggtgatgtggcaaacctagagaatgagtccaaagtggcg

SEQ ID NO: 36 - protein, 745 aa, artificial sequence
  Variant AAV capsid
MAADGYLPDWLEDTLSEGIRQWWKLKPGPPPPKAAERHKDDSRGLVLPGYKYLGPFNGLDKGEPVNEADAAALEHDKAYDRQLDSGDNPYLKYNHADAEFQERLKEDTSFGGNLGRAVFQAKKRVLEPLGLVEEPVKTAPGKKRPVEHSPVEPDSSSGTGKAGQQPARKRLNFGQTGDADSVPDPQPLGQPPAAPSGLGTNTMATGSGAPMADNNEGADGVGNSSGNWHCDSTWMGDRVITTSTRTWALPTYNNHLYKQISSQSGASNDNHYFGYSTPWGYFDFNRFHCHFSPRDWQRLINNNWGFRPKRLNFKLFNIQVKEVTQNDGTTTIANNLTSTVQVFTDSEYQLPYVLGSAHQGCLPPFPADVFMVPQYGYLTLNNGSQAVGRSSFYCLEYFPSQMLRTGNNFTFSYTFEDVPFHSSYAHSQSLDRLMNPLIDQYLYYLSRTNTPSGTTTQSRLQFSQAGASDIRDQSRNWLPGPCYRQQRVSKTSADNNNSEYSWTGATKYHLNGRDSLVNPGPAMASHKDDEEKFFPQSGVLIFGKQGSEKTNVDIEKVMITDEEEIRTTNPVATEQYGSVSTNLQRGNLAISDQTKHARQAATADVNTQGVLPGMVWQDRDVYLQGPIWAKIPHTDGHFHPSPLMGGFGLKHPPPQILIKNTPVPANPSTTFSAAKFASFITQYSTGQVSVEIEWELQKENSKRWNPEIQYTSNYNKSVNVDFTVDTNGVYSEPRPIGTRYLTRNL

SEQ ID NO: 37 - protein, 10 aa, artificial sequence
  insertion peptide
LAISDQTKHA